European Patent Specification EP 3 638 288 B1, published November 13, 2024. Title: METHODS FOR REGULATING FREE FATTY ACID FLUX USING FAT SPECIFIC PROTEIN 27 (FSP27) COMPOSITIONS. Applicant: OHIO UNIVERSITY. Application PCT/US2018/037443. The sequence listing filed with the application follows.

SEQUENCE LISTING (7 sequences)

SEQ ID NO: 1 - DNA, 11 bp, Unknown
  Description of Unknown: Egr1 binding site
ccgccctcacc

SEQ ID NO: 2 - protein, 238 aa, Homo sapiens
MEYAMKSLSLLYPKSLSRHVSVRTSVVTQQLLSEPSPKAPRARPCRVSTADRSVRKGIMAYSLEDLLLKVRDTLMLADKPFFLVLEEDGTTVETEEYFQALAGDTVFMVLQKGQKWQPPSEQGTRHPLSLSHKPAKKIDVARVTFDLYKLNPQDFIGCLNVKATFYDTYSLSYDLHCCGAKRIMKEAFRWALFSMQATGHVLLGTSCYLQQLLDATEEGQPPKGKASSLIPTCLKILQ

SEQ ID NO: 3 - protein, 239 aa, Mus sp.
MDYAMKSLSLLYPRSLSRHVAVSTAVVTQQLVSKPSRETPRARPCRVSTADRKVRKGIMAHSLEDLLNKVQDILKLKDKPFSLVLEEDGTIVETEEYFQALAKDTMFMVLLKGQKWKPPSEQRKKRAQLALSQKPTKKIDVARVTFDLYKLNPQDFIGCLNVKATLYDTYSLSYDLHCYKAKRIVKEMLRWTLFSMQATGHMLLGTSSYMQQFLDATEEEQPAKAKPSSLLPACLKMLQ

SEQ ID NO: 4 - protein, 246 aa, Macaca mulatta
MGSLRKGFGLLKDPWERAGFDWAACLRVSVRTSVVTQQLLSEPSPEAPRARPCRVSTADRSVRKGIMAYSLEDLLLKVRDTLMLADKPFFLVLEEDGTTVETEEYFQALAGDIVFMVLQKGQKWQPPSEQGTRHPQSLSHKPAKKIDVARVTFDLYKLNPQDFIGCLNVKATFYDTYSLSYDLHCCGAKRIVKEALRWALFSMQATGHVMLGTSCYLQQLLDATEEGQPPKGKASSLIPTCLRILQ

SEQ ID NO: 5 - protein, 238 aa, Canis familiaris
MEYAMKSLSLLYPKSLSRHVAVSTSVVTQQLSSKSSLEAPKARPCRVSTADRSVRKGIIAHSLKDLLNKVRDTLLLADKPFYLVLEEDGTTVETEEYFQALADDTVFMVLQKGQKWQPPQEQGSRYQLSLSHKPAKKIDVAQVTFDLYKMNPQDFIGCLNVKATLYGTYSLSYDLHCYGAKRIMKEVLRWALFSMKTTGHVLLGTSCYMQQLLDATEGGQPPEGKARSLIPTSLKMLQ

SEQ ID NO: 6 - protein, 222 aa, Bos taurus
MAMYTAVSTSVVTQQQLSEPSAEAPRARPCRVTTADRSVRKGIMVHSLEDLHVKVQDTLMLAYRPFFLVLEEDGTTVETEEYFQSLADDTVFMVLHKGQKWQPPSEQSTRYQLALSHKPAKIDVAQVTFDLYKVNPQDFIGCLNVKATLYGTYSVSYDLHCSGAKRIMKEALRWALFSMRTTGHMLLGTSCYLQQLLDATEREQPPKSKAASLIPTSLKMLQ

SEQ ID NO: 7 - protein, 236 aa, Xenopus sp.
MEYAMKSLSLLSPKSLTKCVSVSASMTQQLLSRPVSKPRPFRVCNSNRSLRKGIVANSLEDLINKTQDALLMLEAITLVLDEDGTCVDTEEFFRSLDDGAVFMALAKGQKWKPTENSGYHLSLTKKPARKIDVACVSFDLYKNHPRDFIGCLNVKATLYGTYSLSYDLQCYGAKRMVKEALRWTLYTMQATGHVLLGTSCYMKQLLDATERPVTEEEKSSTTLRDFIPFSPWKMLQ